European Patent Application EP 4 534 666 A1, published April 9, 2025. Title: Method and reagent for nucleic acid extraction and purification using porous nanomaterial. Applicant: HANGZHOU NEW HORIZON HEALTH TECHNOLOGY CO. LTD. The sequence listing filed with the application follows.

SEQUENCE LISTING (4 sequences)

SEQ ID NO: 1 - DNA, 44 bp, synthetic construct
  source 1..44: mol_type = other DNA
ctcaactggtgtcgtggagtcggcaattcagttgagaaacccca

SEQ ID NO: 2 - DNA, 18 bp, synthetic construct
  source 1..18: mol_type = other DNA
ttcagttgagaaacccca

SEQ ID NO: 3 - DNA, 19 bp, synthetic construct
  source 1..19: mol_type = other DNA
gccgagtggagtgtgacaa

SEQ ID NO: 4 - DNA, 20 bp, synthetic construct
  source 1..20: mol_type = other DNA
ctcaactggtgtcgtggagt